European Patent Application EP 4 703 465 A1, published March 4, 2026. Title: 一种多能干细胞来源的RPE细胞、制剂、药物组合物、试剂、方法及试剂盒. Applicant: 南京艾尔普再生医学科技有限公司. The sequence listing filed with the application follows.

SEQUENCE LISTING (10 sequences)

SEQ ID NO: 1 - DNA, 21 bp, unidentified
  source 1..21: mol_type = other DNA
ggagcgagatccctccaaaat

SEQ ID NO: 2 - DNA, 23 bp, unidentified
  source 1..23: mol_type = other DNA
ggctgttgtcatacttctcatgg

SEQ ID NO: 3 - DNA, 23 bp, unidentified
  source 1..23: mol_type = other DNA
ttggatctgagccattttaccac

SEQ ID NO: 4 - DNA, 23 bp, unidentified
  source 1..23: mol_type = other DNA
gtcagtaacctctactcctcgaa

SEQ ID NO: 5 - DNA, 19 bp, unidentified
  source 1..19: mol_type = other DNA
tgcccaggcatgaacacac

SEQ ID NO: 6 - DNA, 22 bp, unidentified
  source 1..22: mol_type = other DNA
tgggaaaaatacacgctgtgag

SEQ ID NO: 7 - DNA, 20 bp, unidentified
  source 1..20: mol_type = other DNA
ccagggcaatcggtggtagt

SEQ ID NO: 8 - DNA, 20 bp, unidentified
  source 1..20: mol_type = other DNA
acgggcactcccgcttatac

SEQ ID NO: 9 - DNA, 21 bp, unidentified
  source 1..21: mol_type = other DNA
aactgagcctaccacacaaca

SEQ ID NO: 10 - DNA, 19 bp, unidentified
  source 1..19: mol_type = other DNA
cggattcgacctccaagcc